European Patent Application EP 4 183 881 A1, published May 24, 2023. Title: MUTANT OF PYRUVATE CARBOXYLASE GENE PROMOTER AND USE THEREOF. Applicant: Tianjin Institute of Industrial Biotechnology, Chinese Academy of Sciences. The sequence listing filed with the application follows.

SEQUENCE LISTING (59 sequences)

SEQ ID NO: 1 - DNA, 373 bp, Corynebacterium glutamicum
gaaaacccaggattgctttgtgcactcctgggttttcactttgttaagcagttttggggaaaagtgcaaagtttgcaaagtttagaaatattttaagaggtaagatgtctgcaggtggaagcgtttaaatgcgttaaacttggccaaatgtggcaacctttgcaaggtgaaaaactggggcggggttagatcctggggggtttatttcattcactttggcttgaagtcgtgcaggtcaggggagtgttgcccgaaaacattgagaggaaaacaaaaacctaattttgattcgtactgatttctgctacgatgagtcaacgcagtgactgctatcacccttggcggtctcttgttgaaaggaataattactcta

SEQ ID NO: 2 - DNA, 373 bp, Corynebacterium glutamicum
gaaaacccaggattgctttgtgcactcctgggttttcactttgttaagcagttttggggaaaagtgcaaagtttgcaaagtttagaaatattttaagaggtaagatgtctgcaggtggaagcgtttaaatgcgttaaacttggccaaatgtggcaacctttgcaaggtgaaaaactggggcggggttagatcctggggggtttatttcattcactttggcttgaagtcgtgcaggtcaggggagtgttgcccgaaaacattgagaggaaaacaaaaacggattgttgatttgagcttgatgagcgtacaatcaacttacgcagtgactgctatcacccttggcggtctcttgttgaaaggaataattactcta

SEQ ID NO: 3 - DNA, 373 bp, Corynebacterium glutamicum
gaaaacccaggattgctttgtgcactcctgggttttcactttgttaagcagttttggggaaaagtgcaaagtttgcaaagtttagaaatattttaagaggtaagatgtctgcaggtggaagcgtttaaatgcgttaaacttggccaaatgtggcaacctttgcaaggtgaaaaactggggcggggttagatcctggggggtttatttcattcactttggcttgaagtcgtgcaggtcaggggagtgttgcccgaaaacattgagaggaaaacaaaaacttctccttgattgcgccttaaccgtggtatgattcgataacgcagtgactgctatcacccttggcggtctcttgttgaaaggaataattactcta

SEQ ID NO: 4 - DNA, 373 bp, Corynebacterium glutamicum
gaaaacccaggattgctttgtgcactcctgggttttcactttgttaagcagttttggggaaaagtgcaaagtttgcaaagtttagaaatattttaagaggtaagatgtctgcaggtggaagcgtttaaatgcgttaaacttggccaaatgtggcaacctttgcaaggtgaaaaactggggcggggttagatcctggggggtttatttcattcactttggcttgaagtcgtgcaggtcaggggagtgttgcccgaaaacattgagaggaaaacaaaaacattgatttgattggaaccttactgtgctatgatttggtaacgcagtgactgctatcacccttggcggtctcttgttgaaaggaataattactcta

SEQ ID NO: 5 - DNA, 373 bp, Corynebacterium glutamicum
gaaaacccaggattgctttgtgcactcctgggttttcactttgttaagcagttttggggaaaagtgcaaagtttgcaaagtttagaaatattttaagaggtaagatgtctgcaggtggaagcgtttaaatgcgttaaacttggccaaatgtggcaacctttgcaaggtgaaaaactggggcggggttagatcctggggggtttatttcattcactttggcttgaagtcgtgcaggtcaggggagtgttgcccgaaaacattgagaggaaaacaaaaactcgagtttgatttcacaacgtgtgtgataggatataataacgcagtgactgctatcacccttggcggtctcttgttgaaaggaataattactcta

SEQ ID NO: 6 - DNA, 373 bp, Corynebacterium glutamicum
gaaaacccaggattgctttgtgcactcctgggttttcactttgttaagcagttttggggaaaagtgcaaagtttgcaaagtttagaaatattttaagaggtaagatgtctgcaggtggaagcgtttaaatgcgttaaacttggccaaatgtggcaacctttgcaaggtgaaaaactggggcggggttagatcctggggggtttatttcattcactttggcttgaagtcgtgcaggtcaggggagtgttgcccgaaaacattgagaggaaaacaaaaacttgcgtttgattaaagtatgcaagggctagtatggtgatacgcagtgactgctatcacccttggcggtctcttgttgaaaggaataattactcta

SEQ ID NO: 7 - DNA, 373 bp, Corynebacterium glutamicum
gaaaacccaggattgctttgtgcactcctgggttttcactttgttaagcagttttggggaaaagtgcaaagtttgcaaagtttagaaatattttaagaggtaagatgtctgcaggtggaagcgtttaaatgcgttaaacttggccaaatgtggcaacctttgcaaggtgaaaaactggggcggggttagatcctggggggtttatttcattcactttggcttgaagtcgtgcaggtcaggggagtgttgcccgaaaacattgagaggaaaacaaaaacatcattttgattccggcgcacatgtggtaatatggtattacgcagtgactgctatcacccttggcggtctcttgttgaaaggaataattactcta

SEQ ID NO: 8 - DNA, 373 bp, Corynebacterium glutamicum
gaaaacccaggattgctttgtgcactcctgggttttcactttgttaagcagttttggggaaaagtgcaaagtttgcaaagtttagaaatattttaagaggtaagatgtctgcaggtggaagcgtttaaatgcgttaaacttggccaaatgtggcaacctttgcaaggtgaaaaactggggcggggttagatcctggggggtttatttcattcactttggcttgaagtcgtgcaggtcaggggagtgttgcccgaaaacattgagaggaaaacaaaaactcgccattgattgcccgccatccatgctataatcggaagacgcagtgactgctatcacccttggcggtctcttgttgaaaggaataattactcta

SEQ ID NO: 9 - DNA, 373 bp, Corynebacterium glutamicum
gaaaacccaggattgctttgtgcactcctgggttttcactttgttaagcagttttggggaaaagtgcaaagtttgcaaagtttagaaatattttaagaggtaagatgtctgcaggtggaagcgtttaaatgcgttaaacttggccaaatgtggcaacctttgcaaggtgaaaaactggggcggggttagatcctggggggtttatttcattcactttggcttgaagtcgtgcaggtcaggggagtgttgcccgaaaacattgagaggaaaacaaaaacttccgcttgattgtggccatagtatgatattattaattaacgcagtgactgctatcacccttggcggtctcttgttgaaaggaataattactcta

SEQ ID NO: 10 - DNA, 373 bp, Corynebacterium glutamicum
gaaaacccaggattgctttgtgcactcctgggttttcactttgttaagcagttttggggaaaagtgcaaagtttgcaaagtttagaaatattttaagaggtaagatgtctgcaggtggaagcgtttaaatgcgttaaacttggccaaatgtggcaacctttgcaaggtgaaaaactggggcggggttagatcctggggggtttatttcattcactttggcttgaagtcgtgcaggtcaggggagtgttgcccgaaaacattgagaggaaaacaaaaaccggatcttgattttatgatgggtattgtataatcttggtacgcagtgactgctatcacccttggcggtctcttgttgaaaggaataattactcta

SEQ ID NO: 11 - DNA, 373 bp, Corynebacterium glutamicum
gaaaacccaggattgctttgtgcactcctgggttttcactttgttaagcagttttggggaaaagtgcaaagtttgcaaagtttagaaatattttaagaggtaagatgtctgcaggtggaagcgtttaaatgcgttaaacttggccaaatgtggcaacctttgcaaggtgaaaaactggggcggggttagatcctggggggtttatttcattcactttggcttgaagtcgtgcaggtcaggggagtgttgcccgaaaacattgagaggaaaacaaaaaccggatattgatttggccggtgttgtggtagtatcgtgttacgcagtgactgctatcacccttggcggtctcttgttgaaaggaataattactcta

SEQ ID NO: 12 - DNA, 373 bp, Corynebacterium glutamicum
gaaaacccaggattgctttgtgcactcctgggttttcactttgttaagcagttttggggaaaagtgcaaagtttgcaaagtttagaaatattttaagaggtaagatgtctgcaggtggaagcgtttaaatgcgttaaacttggccaaatgtggcaacctttgcaaggtgaaaaactggggcggggttagatcctggggggtttatttcattcactttggcttgaagtcgtgcaggtcaggggagtgttgcccgaaaacattgagaggaaaacaaaaacaggggtttgattggccgctcggtgtgttatcatggagagacgcagtgactgctatcacccttggcggtctcttgttgaaaggaataattactcta

SEQ ID NO: 13 - DNA, 373 bp, Corynebacterium glutamicum
gaaaacccaggattgctttgtgcactcctgggttttcactttgttaagcagttttggggaaaagtgcaaagtttgcaaagtttagaaatattttaagaggtaagatgtctgcaggtggaagcgtttaaatgcgttaaacttggccaaatgtggcaacctttgcaaggtgaaaaactggggcggggttagatcctggggggtttatttcattcactttggcttgaagtcgtgcaggtcaggggagtgttgcccgaaaacattgagaggaaaacaaaaacgagttgttgatttcgttggtgcacgtatacaatggttttacgcagtgactgctatcacccttggcggtctcttgttgaaaggaataattactcta

SEQ ID NO: 14 - DNA, 373 bp, Corynebacterium glutamicum
gaaaacccaggattgctttgtgcactcctgggttttcactttgttaagcagttttggggaaaagtgcaaagtttgcaaagtttagaaatattttaagaggtaagatgtctgcaggtggaagcgtttaaatgcgttaaacttggccaaatgtggcaacctttgcaaggtgaaaaactggggcggggttagatcctggggggtttatttcattcactttggcttgaagtcgtgcaggtcaggggagtgttgcccgaaaacattgagaggaaaacaaaaaccttggcttgatttttgtttgagggttgtataatgttattacgcagtgactgctatcacccttggcggtctcttgttgaaaggaataattactcta

SEQ ID NO: 15 - DNA, 373 bp, Corynebacterium glutamicum
gaaaacccaggattgctttgtgcactcctgggttttcactttgttaagcagttttggggaaaagtgcaaagtttgcaaagtttagaaatattttaagaggtaagatgtctgcaggtggaagcgtttaaatgcgttaaacttggccaaatgtggcaacctttgcaaggtgaaaaactggggcggggttagatcctggggggtttatttcattcactttggcttgaagtcgtgcaggtcaggggagtgttgcccgaaaacattgagaggaaaacaaaaacgactagttgatttccgcccttggttgatattatgcttgaacgcagtgactgctatcacccttggcggtctcttgttgaaaggaataattactcta

SEQ ID NO: 16 - DNA, 373 bp, Corynebacterium glutamicum
gaaaacccaggattgctttgtgcactcctgggttttcactttgttaagcagttttggggaaaagtgcaaagtttgcaaagtttagaaatattttaagaggtaagatgtctgcaggtggaagcgtttaaatgcgttaaacttggccaaatgtggcaacctttgcaaggtgaaaaactggggcggggttagatcctggggggtttatttcattcactttggcttgaagtcgtgcaggtcaggggagtgttgcccgaaaacattgagaggaaaacaaaaacatccgcttgatttaggcgtacgtttaatagtatattgaaacgcagtgactgctatcacccttggcggtctcttgttgaaaggaataattactcta

SEQ ID NO: 17 - DNA, 373 bp, Corynebacterium glutamicum
gaaaacccaggattgctttgtgcactcctgggttttcactttgttaagcagttttggggaaaagtgcaaagtttgcaaagtttagaaatattttaagaggtaagatgtctgcaggtggaagcgtttaaatgcgttaaacttggccaaatgtggcaacctttgcaaggtgaaaaactggggcggggttagatcctggggggtttatttcattcactttggcttgaagtcgtgcaggtcaggggagtgttgcccgaaaacattgagaggaaaacaaaaaccggggcttgatttccttgtcgtggcgttattataatggaacgcagtgactgctatcacccttggcggtctcttgttgaaaggaataattactcta

SEQ ID NO: 18 - DNA, 373 bp, Corynebacterium glutamicum
gaaaacccaggattgctttgtgcactcctgggttttcactttgttaagcagttttggggaaaagtgcaaagtttgcaaagtttagaaatattttaagaggtaagatgtctgcaggtggaagcgtttaaatgcgttaaacttggccaaatgtggcaacctttgcaaggtgaaaaactggggcggggttagatcctggggggtttatttcattcactttggcttgaagtcgtgcaggtcaggggagtgttgcccgaaaacattgagaggaaaacaaaaacatggagttgattatacgatactacagatactatactggtacgcagtgactgctatcacccttggcggtctcttgttgaaaggaataattactcta

SEQ ID NO: 19 - DNA, 373 bp, Corynebacterium glutamicum
gaaaacccaggattgctttgtgcactcctgggttttcactttgttaagcagttttggggaaaagtgcaaagtttgcaaagtttagaaatattttaagaggtaagatgtctgcaggtggaagcgtttaaatgcgttaaacttggccaaatgtggcaacctttgcaaggtgaaaaactggggcggggttagatcctggggggtttatttcattcactttggcttgaagtcgtgcaggtcaggggagtgttgcccgaaaacattgagaggaaaacaaaaacccgtagttgattgacttgggcagtatatagtataatgaaacgcagtgactgctatcacccttggcggtctcttgttgaaaggaataattactcta

SEQ ID NO: 20 - DNA, 373 bp, Corynebacterium glutamicum
gaaaacccaggattgctttgtgcactcctgggttttcactttgttaagcagttttggggaaaagtgcaaagtttgcaaagtttagaaatattttaagaggtaagatgtctgcaggtggaagcgtttaaatgcgttaaacttggccaaatgtggcaacctttgcaaggtgaaaaactggggcggggttagatcctggggggtttatttcattcactttggcttgaagtcgtgcaggtcaggggagtgttgcccgaaaacattgagaggaaaacaaaaaccgggccttgattgtaagataagacatttagtataattagacgcagtgactgctatcacccttggcggtctcttgttgaaaggaataattactcta

SEQ ID NO: 21 - DNA, 373 bp, Corynebacterium glutamicum
gaaaacccaggattgctttgtgcactcctgggttttcactttgttaagcagttttggggaaaagtgcaaagtttgcaaagtttagaaatattttaagaggtaagatgtctgcaggtggaagcgtttaaatgcgttaaacttggccaaatgtggcaacctttgcaaggtgaaaaactggggcggggttagatcctggggggtttatttcattcactttggcttgaagtcgtgcaggtcaggggagtgttgcccgaaaacattgagaggaaaacaaaaaccgatgtttgattgggggaatcgggggttacgatactaggacgcagtgactgctatcacccttggcggtctcttgttgaaaggaataattactcta

SEQ ID NO: 22 - DNA, 42 bp, Artificial Sequence
  Primer Sequence
cctgatgcggtattttctccgaaaacccaggattgctttgtg

SEQ ID NO: 23 - DNA, 23 bp, Artificial Sequence
  Primer Sequence
gcggacagcttcagaagcaaaag

SEQ ID NO: 24 - DNA, 84 bp, Artificial Sequence
  Primer Sequence
ttgcttctgaagctgtccgcggcggtggctctggaggtggtgggtccggcggtggctctgcttcctccgaagacgttatcaaag

SEQ ID NO: 25 - DNA, 21 bp, Artificial Sequence
  Primer Sequence
ggagaaaataccgcatcaggc

SEQ ID NO: 26 - DNA, 89 bp, Artificial Sequence
  Primer Sequence
cccgaaaacattgagaggaaaacaaaaacnnnnnnttgattnnnnnnnnnnnnnnntannatnnnnnnacgcagtgactgctatcaccc

SEQ ID NO: 27 - DNA, 25 bp, Artificial Sequence
  Primer Sequence
aaccttccatacgaactttgaaacg

SEQ ID NO: 28 - DNA, 23 bp, Artificial Sequence
  Primer Sequence
caaagttcgtatggaaggttccg

SEQ ID NO: 29 - DNA, 21 bp, Artificial Sequence
  Primer Sequence
ttcctctcaatgttttcgggc

SEQ ID NO: 30 - DNA, 43 bp, Artificial Sequence
  Primer Sequence
caggaaacagctatgacatggtatcgccatgtatcacgcactc

SEQ ID NO: 31 - DNA, 46 bp, Artificial Sequence
  Primer Sequence
tcagtacgaatcaaaattaggtttttgttttcctctcaatgttttc

SEQ ID NO: 32 - DNA, 46 bp, Artificial Sequence
  Primer Sequence
atggccacaatcaagcggaagtttttgttttcctctcaatgttttc

SEQ ID NO: 33 - DNA, 46 bp, Artificial Sequence
  Primer Sequence
tacgcctaaatcaagcggatgtttttgttttcctctcaatgttttc

SEQ ID NO: 34 - DNA, 46 bp, Artificial Sequence
  Primer Sequence
tatcttacaatcaaggcccggtttttgttttcctctcaatgttttc

SEQ ID NO: 35 - DNA, 60 bp, Artificial Sequence
  Primer Sequence
ctaattttgattcgtactgatttctgctacgatgagtcaacgcagtgactgctatcaccc

SEQ ID NO: 36 - DNA, 60 bp, Artificial Sequence
  Primer Sequence
ttccgcttgattgtggccatagtatgatattattaattaacgcagtgactgctatcaccc

SEQ ID NO: 37 - DNA, 60 bp, Artificial Sequence
  Primer Sequence
atccgcttgatttaggcgtacgtttaatagtatattgaaacgcagtgactgctatcaccc

SEQ ID NO: 38 - DNA, 60 bp, Artificial Sequence
  Primer Sequence
cgggccttgattgtaagataagacatttagtataattagacgcagtgactgctatcaccc

SEQ ID NO: 39 - DNA, 44 bp, Artificial Sequence
  Primer Sequence
tgtaaaacgacggccagtgcctaatttgcgaagctcatcaggtg

SEQ ID NO: 40 - DNA, 19 bp, Artificial Sequence
  Primer Sequence
gcactggccgtcgttttac

SEQ ID NO: 41 - DNA, 24 bp, Artificial Sequence
  Primer Sequence
catgtcatagctgtttcctgtgtg

SEQ ID NO: 42 - DNA, 21 bp, Artificial Sequence
  Primer Sequence
ggagaaaataccgcatcaggc

SEQ ID NO: 43 - DNA, 22 bp, Artificial Sequence
  Primer Sequence
ctgttttggcggatgagagaag

SEQ ID NO: 44 - DNA, 42 bp, Artificial Sequence; identical to SEQ ID NO: 22
  Primer Sequence

SEQ ID NO: 45 - DNA, 47 bp, Artificial Sequence
  Primer Sequence
ttggagatgcgctcacgcattagagtaattattcctttcaacaagag

SEQ ID NO: 46 - DNA, 21 bp, Artificial Sequence
  Primer Sequence
atgcgtgagcgcatctccaac

SEQ ID NO: 47 - DNA, 22 bp, Artificial Sequence
  Primer Sequence
ttacgcgcggctggcgtagttg

SEQ ID NO: 48 - DNA, 42 bp, Artificial Sequence
  Primer Sequence
actacgccagccgcgcgtaagccttttatggtgtgatccgac

SEQ ID NO: 49 - DNA, 24 bp, Artificial Sequence
  Primer Sequence
ttaaggcctaatttgtcctgtgcc

SEQ ID NO: 50 - DNA, 39 bp, Artificial Sequence
  Primer Sequence
caggacaaattaggccttaatttgtcgttttgggccccc

SEQ ID NO: 51 - DNA, 43 bp, Artificial Sequence
  Primer Sequence
tctctcatccgccaaaacagctagcgctttccgagttcttcag

SEQ ID NO: 52 - DNA, 42 bp, Artificial Sequence
  Primer Sequence
caggaaacagctatgacatgttctagggcatcgacgaaccag

SEQ ID NO: 53 - DNA, 22 bp, Artificial Sequence
  Primer Sequence
gaaattgttaaaagcgcagcgc

SEQ ID NO: 54 - DNA, 42 bp, Artificial Sequence
  Primer Sequence
gctgcgcttttaacaatttcgaaaacccaggattgctttgtg

SEQ ID NO: 55 - DNA, 21 bp, Artificial Sequence
  Primer Sequence
tcgaagccgcacgtcatctag

SEQ ID NO: 56 - DNA, 42 bp, Artificial Sequence
  Primer Sequence
tagatgacgtgcggcttcgatccgtgaacgcctatctgtacg

SEQ ID NO: 57 - DNA, 40 bp, Artificial Sequence
  Primer Sequence
tgtaaaacgacggccagtgcgatcgattccacgcccaaac

SEQ ID NO: 58 - DNA, 19 bp, Artificial Sequence
  Primer Sequence
gcactggccgtcgttttac

SEQ ID NO: 59 - DNA, 24 bp, Artificial Sequence
  Primer Sequence
catgtcatagctgtttcctgtgtg